European Patent Application EP 4 632 073 A1, published October 15, 2025. Title: Microorganism having retinoid producing ability with attenuated activity of chitin transglycosylase and method for producing retinoid using the same. Applicant: CJ CheilJedang Corporation. The sequence listing filed with the application follows.

SEQUENCE LISTING (43 sequences)

SEQ ID NO: 1 - protein, 515 aa, Yarrowia lipolytica
MFKALTTFLLATTALGQTYSTCNPLTQTCKPDPALGGAKMFDFTQEQGDWHVTFKPDRVEYTPEGVSLRVQTQGDNPTLQSDFYLMFGRVEAVIQAAPGVGIVSSFVLQSDDLDEIDLEWLGGDNTQVQTNFFVKGNTDTYDRGQFHGIGNPTGQFHTYVIEWTSEQITWTINGQVVRTLLSNDWHGFPQSPMNIRMGVWAGGDPTNNPGTIQWAGGETNYQTGPYPMLIKSVNVEDYSTGDAYEYSDRSGTWQSIKAQNGEVHPVRPAVIPPADGSKFDLVSADQGDKPSTGALQASSTQASPEASSQAPSEAPSEASSKTSSEASSVQATPSVEPTSSIPAPSTSAASSAASSAAPTTSSTLSIPVLVPGPAKNTSSAVSSSTNSSTPVTTHVTKPANRTSSTVFATVTSCKDDACKKTEVPKPVANSTVATSKPASKPASKTVLPVTSVAPTTSKPVPTQTKTEAESSASVSGVPTISQATASTTAHQANTGVVTEASFGAIAVAAFALMLI

SEQ ID NO: 2 - protein, 584 aa, Yarrowia lipolytica
MRLSLSVVASLAMSVMAQTYTDCNPLHETCPADKALGTSKSFDFTQGPSDDFPPSFKPHRITYSNDTGVSLAVVEQGDNPTIQSDFYIMFGRVEAVVQAAPGQGIISSVVLQSDDLDEIDLEWIGGDANNVQTNFYIQGNTTTYDRGAIHPVANSNSEFHTYTVEWTKDDLTWFIDGEAVRTVPSTFSQGYPQSPMNIRIGVWAGGDPTNNAGVIEWAGGETDYTKSPYPMYVKSVNVQDYSTGSEYSYSDHSGTWESIVAKDGEVNANAPVEEVPEETTSAVESSIPVETSAAVESSAVESSAVESSAVESSAPITSAPAPVSSAPAFTNSTISTGVSSGAVVTVEATEHVESTLTKTVTHCEDNKCVSKPQPTVTVTKHCTLDKCVSKTIPVEYVTVTATTTKVVTEICPEAKCHKISSVPVRPAPTEAPLKPTNLKTTQTVTKTGTVVVKTDTPKSEPASEVSKPTTESKPTAESKPTAESKPVAKPTGSSPVEVPAEGKSTQTIHLTQIVTIGTQTVQTVIPQSDIPTAAPQTSPVVQVNNGTVPQVPQAPNTFPAQANGAASKAVSVVAAMVAMVALLI

SEQ ID NO: 3 - protein, 515 aa, Yarrowia lipolytica
MKLSTLVLAALTAVAVADDYKSISCDVDNHCPEDKPCCSQYGECGTGAYCLGGCDPKSSFELKSCMPMPVCKKRQSKFTSMDRIAKNTEYLGDAENFDWVYTGNLIQQNNGLLLTMPKNSVGTVLSSTDYMWYGKVSATFKSSHLQGVVSAFILFSDVKDEIDYEFVGADVNTVQTNYYWQGVLDWTHGINISVDNTHENFFTYSIDWTPDQITWAVDDQPGRVLKKSDTWDEKTKSYMYPQTPSRIQLSLWPAGQASNAEGTIAWAGGEIDWDAEDIQKYGYYYATVTEIDVDCYDPPASAKKSGDKSYRYTDLNAMEADVEITGDDTVLASFDATGADPEKDDGSKNGTAPTGMMQHPDNDPNIANVTGGVAASTKKTTSVASSTESLEDVSGSAIKKSTSSKESTSSDADPTEVVSGERVSSKETSSASASSGNNNGGNNNNGGNSGSAAATGSSSRNPQGNAATASNTGNGGFQQFGQASGSAAEKANTAGSNGMSSLLLAGALAAASLLM

SEQ ID NO: 4 - DNA, 1548 bp, Yarrowia lipolytica
  source 1..1548: mol_type = genomic DNA
atgttcaaggctctgaccaccttcctgctggccacaaccgccctgggccagacatactccacctgcaacccgctgacacaaacgtgtaagccggacccggcgctgggcggagccaagatgttcgacttcacccaggaacagggcgactggcacgtgaccttcaagcccgaccgggtcgaatacacccccgagggagtgtctctgcgggtccagacccagggcgacaaccccacgctgcagtctgacttttatctcatgtttggccgtgtcgaggccgtgatccaggcagctcccggcgtgggcatcgtgtcctcctttgtgctgcagagcgacgacctcgatgagatcgacctcgagtggctcggaggcgacaacacccaggtccagacaaacttctttgtcaagggaaacacagacacctacgatcgaggccagttccatggcattggcaaccccacgggccaattccacacctacgtcattgagtggacctccgaacagatcacctggaccatcaacggccaggtggtccgaaccctgctctccaacgattggcatggcttcccccagtcacccatgaacatccgaatgggcgtctgggctggaggagaccccaccaacaaccccggaaccatccagtgggccggaggagaaaccaactaccagaccggtccttaccccatgctcatcaagtccgttaacgtcgaggattactctaccggtgatgcttacgagtattctgatcgatccggaacctggcagtccatcaaggcacagaacggagaggttcatcccgttcgacctgccgtgattcctcctgccgatggctccaagtttgatcttgtttctgccgaccagggtgataagcctagcactggagctctgcaagcttcttccacccaggcttctcccgaggcttcttctcaggctccttctgaggctccttctgaggcttcttccaagacttcttctgaggcttcttccgttcaggctaccccttctgtcgagcctacttcttctattcccgctccttctacatctgctgcctcttctgctgcctcttctgcggctcccactacctcttccaccctctccatccctgtgttggtgcctggacctgctaagaacacctcctccgcagtgtcttcttctaccaacagctcaactcccgtgaccacccacgtgaccaagccggccaaccgaaccagctccaccgtgttcgccaccgtcacttcctgcaaggacgatgcctgcaagaagactgaggtgcccaaacccgtggccaactctaccgtggccacctccaagcctgcttccaagcccgcttccaagaccgtccttcctgtgacctctgtggctcccaccacctccaagcctgtccccactcagaccaagactgaggccgagtcttctgcttctgtttctggcgtccccacaatttctcaggccactgcctccaccaccgctcaccaggccaacactggagttgtcactgaggcttctttcggcgccattgccgttgctgcctttgctctgatgctcatttaa

SEQ ID NO: 5 - DNA, 1755 bp, Yarrowia lipolytica
  source 1..1755: mol_type = genomic DNA
atgcgactttctctttccgttgtggcctccttggccatgtctgttatggcccagacttacaccgattgcaaccctctgcacgagacctgtcccgccgataaggctcttggaacctccaagtccttcgatttcacccagggtccctccgacgacttccctccttccttcaagccccaccgaatcacctactccaacgacactggtgtttctctggctgttgttgagcagggcgacaaccccaccattcagtccgacttttacatcatgtttggccgagttgaggccgtggtccaggccgcccctggtcagggaatcatctcgtctgtggttctccagtccgacgatctcgatgagattgatctggaatggattggaggagatgctaacaacgtacagactaacttctacatccagggtaacaccaccacttacgaccgaggtgccatccaccccgtcgctaactccaactccgagttccacacctacactgttgagtggaccaaggatgaccttacctggttcattgacggagaggccgtccgaaccgtgccttccaccttttctcagggatacccccagtctcctatgaacatccgaattggcgtgtgggccggaggagaccccaccaacaacgctggcgtcattgagtgggccggcggagagaccgattacaccaagagcccctaccccatgtacgtcaagtctgtgaacgtccaggactactccactggatccgagtactcctactctgaccactctggaacctgggagtccattgtcgccaaggacggtgaagttaacgctaacgctcctgttgaggaggtgcctgaggagactacttctgccgtggagtcttccattcctgttgagacctccgctgctgtcgagtcttctgctgtcgagtcttctgctgtcgagtcttctgctgtcgagtcttctgctcccatcacttctgctcctgctcccgtctcctctgctcccgccttcaccaactccaccatctccaccggtgtttcttccggcgctgttgtcaccgttgaggccaccgagcacgtcgagtccaccttgaccaagaccgtcacccactgcgaggacaacaagtgcgtctctaagcctcagcctactgtgacagtcaccaagcactgcaccctggacaagtgtgtttctaagaccatccccgtcgagtacgttaccgtcaccgccactaccaccaaggtggtgaccgagatctgccccgaggccaagtgccacaagatctcatctgtccccgttagacctgctcctactgaggctcctctcaagcccaccaacctcaagaccactcagactgttaccaagactggaactgttgttgttaagaccgatacccccaagtctgagcctgcctctgaggtttccaagcccactaccgagtccaagcccactgccgagtccaagcccactgctgagtccaagcccgttgctaagcccactggctcttctcccgtcgaggttcccgctgagggtaagtctacccagactatccacctgacccagattgtcaccattggaacccagaccgtccagactgttatcccccagtctgacatccccaccgctgctccccagacttctcccgtcgtccaggtcaacaacggtaccgtccctcaggtcccccaggctcccaacaccttccctgcccaggctaacggagctgcctccaaggccgtctccgtggtcgccgctatggtcgccatggttgccctgctcatttaa

SEQ ID NO: 6 - DNA, 1548 bp, Yarrowia lipolytica
  source 1..1548: mol_type = genomic DNA
atgaaactctctaccttggtactggccgctctgaccgcggttgccgtggctgatgactacaagtccatctcctgtgacgtggataaccactgtcccgaagacaagccctgctgctctcagtacggtgaatgtggtaccggcgcttactgcctcggaggctgtgaccccaagtcttccttcgagctcaagtcctgtatgcccatgcccgtctgcaagaagcgacagagcaagttcacttccatggatcgaatcgcaaagaacactgagtacctcggagacgccgagaacttcgactgggtctacaccggtaacttgattcagcagaacaacggtttgcttctgaccatgcccaagaactctgtcggaaccgtgctctcctccaccgactacatgtggtatggtaaggtttccgcaaccttcaagtcttctcacctgcagggtgttgtttcggccttcattctcttctccgatgtcaaggatgagatcgattacgagtttgttggtgccgatgtcaacactgttcagaccaactactactggcagggagtgctcgactggactcacggaataaacatttctgtcgataacactcacgagaatttcttcacttactccatcgactggactcccgaccagatcacctgggctgttgacgaccaacctggtcgagttctcaagaagtccgatacctgggacgaaaagaccaagtcttacatgtacccccagactccctctcgaatccagctgtctctgtggcccgctggacaggcctctaacgccgagggaaccattgcctgggccggaggagagattgactgggacgctgaagatatccagaaatacggatactactacgcgactgtcaccgagatcgatgtcgactgttacgatccccccgcttctgccaagaagtctggagacaagtcttaccgatacaccgacctgaacgccatggaggccgatgtcgagattaccggtgatgatactgtcctcgcttctttcgacgctactggtgctgaccctgagaaggacgacggatccaagaacggaactgctcccaccggtatgatgcaacaccccgacaacgaccctaacattgctaacgtcactggtggtgtcgcagccagcacgaagaagaccacatccgtggcttcttctaccgagtccctggaggacgtgtctggttccgccatcaagaagtctacttcttccaaggagtccacctcttctgacgctgaccctaccgaggttgtttctggtgagcgagtttcctccaaggagaccagctctgcttctgcctcttctggcaacaacaacggcggcaacaacaacaacggcggcaacagcggttctgcagctgccaccggctcttcttctcgaaaccctcaaggtaacgctgccaccgcttcaaacaccggaaacggtggcttccaacagttcggccaggcctctggctctgctgctgaaaaggccaacaccgctggctcgaacggtatgtcttcacttctcttggccggagctctggctgctgcctctctgctcatgtaa

SEQ ID NO: 7 - protein, 673 aa, synthetic construct
MTALAYYQIHLIYTLPILGLLGLLTSPILTKFDIYKISILVFIAFSATTPWDSWIIRNGAWTYPSAESGQGVFGTFLDVPYEEYAFFVIQTVITGLVYVLATRHLLPSLALPKTRSSALSLALKALIPLPIIYLFTAHPSPSPDPLVTDHYFYMRALSLLITPPTMLLAALSGEYAFDWKSGRAKSTIAAIMIPTVYLIWVDYVAVGQDSWSINDEKIVGWRLGGVLPIEEAMFFLLTNLMIVLGLSACDHTQALYLLHGRTIYGNKKMPSSFPLITPPVLSLFFSSRPYSSQPKRDLELAVKLLEEKSRSFFVASAGFPSEVRERLVGLYAFCRVTDDLIDSPEVSSNPHATIDMVSDFLTLLFGPPLHPSQPDKILSSPLLPPSHPSRPTGMYPLPPPPSLSPAELVQFLTERVPVQYHFAFRLLAKLQGLIPRYPLDELLRGYTTDLIFPLSTEAVQARKTPIETTADLLDYGLCVAGSVAELLVYVSWASAPSQVPATIEEREAVLVASREMGTALQLVNIARDIKGDATEGRFYLPLSFFGLRDESKLAIPTDWTEPRPQDFDKLLSLSPSSTLPSSNASESFRFEWKTYSLPLVAYAEDLAKHSYKGIDRLPTEVQAGMRAACASYLLIGREIKVVWKGDVGERRTVAGWRRVRKVLSVVMSGWEGQ

SEQ ID NO: 8 - protein, 582 aa, synthetic construct
MGKEQDQDKPTAIIVGCGIGGIATAARLAKEGFQVTVFEKNDYSGGRCSLIERDGYRFDQGPSLLLLPDLFKQTFEDLGEKMEDWVDLIKCEPNYVCHFHDEETFTLSTDMALLKREVERFEGKDGFDRFLSFIQEAHRHYELAVVHVLQKNFPGFAAFLRLQFIGQILALHPFESIWTRVCRYFKTDRLRRVFSFAVMYMGQSPYSAPGTYSLLQYTELTEGIWYPRGGFWQVPNTLLQIVKRNNPSAKFNFNAPVSQVLLSPAKDRATGVRLESGEEHHADVVIVNADLVYASEHLIPDDARNKIGQLGEVKRSWWADLVGGKKLKGSCSSLSFYWSMDRIVDGLGGHNIFLAEDFKGSFDTIFEELGLPADPSFYVNVPSRIDPSAAPEGKDAIVILVPCGHIDASNPQDYNKLVARARKFVIHTLSAKLGLPDFEKMIVAEKVHDAPSWEKEFNLKDGSILGLAHNFMQVLGFRPSTRHPKYDKLFFVGASTHPGTGVPIVLAGAKLTANQVLESFDRSPAPDPNMSLSVPYGKPLKSNGTGIDSQVQLKFMDLERWVYLLVLLIGAVIARSVGVLAF

SEQ ID NO: 9 - DNA, 2022 bp, synthetic construct
  source 1..2022: mol_type = other DNA
atgacggctctcgcatattaccagatccatctgatctatactctcccaattcttggtcttctcggcctgctcacttccccgattttgacaaaatttgacatctacaaaatatcgatcctcgtatttattgcgtttagtgcaaccacaccatgggactcatggatcatcagaaatggcgcatggacatatccatcagcggagagtggccaaggcgtgtttggaacgtttctagatgttccatatgaagagtacgctttctttgtcattcaaaccgtaatcaccggcttggtctacgtcttggcaactaggcaccttctcccatctctcgcgcttcccaagactagatcgtccgccctttctctcgcgctcaaggcgctcatccctctgcccattatctacctatttaccgctcaccccagcccatcgcccgacccgctcgtgacagatcactacttctacatgcgggcactctccttactcatcaccccacctaccatgctcttggcagcattatcaggcgaatatgctttcgattggaaaagtggccgagcaaagtcaactattgcagcaatcatgatcccgacggtgtatctgatttgggtagattatgttgctgtcggtcaagactcttggtcgatcaacgatgagaagattgtagggtggaggcttggaggtgtactacccattgaggaagctatgttcttcttactgacgaatctaatgattgttctgggtctgtctgcctgcgatcatactcaggccctatacctgctacacggtcgaactatttatggcaacaaaaagatgccatcttcatttcccctcattacaccgcctgtgctctccctgttttttagcagccgaccatactcttctcagccaaaacgtgacttggaactggcagtcaagttgttggaggaaaagagccggagcttttttgttgcctcggctggatttcctagcgaagttagggagaggctggttggactatacgcattctgccgggtgactgatgatcttatcgactctcctgaagtatcttccaacccgcatgccacaattgacatggtctccgattttcttaccctactatttgggcccccgctacacccttcgcaacctgacaagatcctttcttcgcctttacttcctccttcgcacccttcccgacccacgggaatgtatcccctcccgcctcctccttcgctctcgcctgccgagctcgttcaattccttaccgaaagggttcccgttcaataccatttcgccttcaggttgctcgctaagttgcaagggctgatccctcgatacccactcgacgaactccttagaggatacaccactgatcttatctttcccttatcgacagaggcagtccaggctcggaagacgcctatcgagaccacagctgacttgctggactatggtctatgtgtagcaggctcagtcgccgagctattggtctatgtctcttgggcaagtgcaccaagtcaggtccctgccaccatagaagaaagagaagctgtgttagtggcaagccgagagatgggaactgcccttcagttggtgaacattgctagggacattaaaggggacgcaacagaagggagattttacctaccactctcattctttggtcttcgggatgaatcaaagcttgcgatcccgactgattggacggaacctcggcctcaagatttcgacaaactcctcagtctatctccttcgtccacattaccatcttcaaacgcctcagaaagcttccggttcgaatggaagacgtactcgcttccattagtcgcctacgcagaggatcttgccaaacattcttataagggaattgaccgacttcctaccgaggttcaagcgggaatgcgagcggcttgcgcgagctacctactgatcggccgagagatcaaagtcgtttggaaaggagacgtcggagagagaaggacagttgccggatggaggagagtacggaaagtcttgagtgtggtcatgagcggatgggaagggcagtaa

SEQ ID NO: 10 - DNA, 1749 bp, synthetic construct
  source 1..1749: mol_type = other DNA
atgggaaaagaacaagatcaggataaacccacagctatcatcgtgggatgtggtatcggtggaatcgccactgccgctcgtcttgctaaagaaggtttccaggtcacggtgttcgagaagaacgactactccggaggtcgatgctctttaatcgagcgagatggttatcgattcgatcaggggcccagtttgctgctcttgccagatctcttcaagcagacattcgaagatttgggagagaagatggaagattgggtcgatctcatcaagtgtgaacccaactatgtttgccacttccacgatgaagagactttcactctttcaaccgacatggcgttgctcaagcgggaagtcgagcgttttgaaggcaaagatggatttgatcggttcttgtcgtttatccaagaagcccacagacattacgagcttgctgtcgttcacgtcctgcagaagaacttccctggcttcgcagcattcttacggctacagttcattggccaaatcctggctcttcaccccttcgagtctatctggacaagagtttgtcgatatttcaagaccgacagattacgaagagtcttctcgtttgcagtgatgtacatgggtcaaagcccatacagtgcgcccggaacatattccttgctccaatacaccgaattgaccgagggcatctggtatccgagaggaggcttttggcaggttcctaatactcttcttcagatcgtcaagcgcaacaatccctcagccaagttcaatttcaacgctccagtttcccaggttcttctctctcctgccaaggaccgagcgactggtgttcgacttgaatccggcgaggaacatcacgccgatgttgtgattgtcaatgctgacctcgtttacgcctccgagcacttgattcctgacgatgccagaaacaagattggccaactgggtgaagtcaagagaagttggtgggctgacttagttggtggaaagaagctcaagggaagttgcagtagtttgagcttctactggagcatggaccgaatcgtggacggtctgggcggacacaatatcttcttggccgaggacttcaagggatcattcgacacaatcttcgaggagttgggtctcccagccgatccttccttttacgtgaacgttccctcgcgaatcgatccttctgccgctcccgaaggcaaagatgctatcgtcattcttgtgccgtgtggccatatcgacgcttcgaaccctcaagattacaacaagcttgttgctcgggcaaggaagtttgtgatccacacgctttccgccaagcttggacttcccgactttgaaaaaatgattgtggcagagaaggttcacgatgctccctcttgggagaaagaattcaacctcaaggacggaagcatcttgggactggctcacaactttatgcaagttcttggtttcaggccgagcaccagacatcccaagtatgacaagttgttctttgtcggggcttcgactcatcccggaactggggttcccatcgtcttggctggagccaagttaactgccaaccaagttctcgaatcctttgaccgatccccagctccagatcccaatatgtcactctccgtaccatatggaaaacctctcaaatcaaatggaacgggtatcgattctcaggtccagctgaagttcatggatttggagagatgggtataccttttggtgttgttgattggggccgtgatcgctcgatccgttggtgttcttgctttctga

SEQ ID NO: 11 - protein, 275 aa, synthetic construct [sequence omitted]

SEQ ID NO: 12 - DNA, 828 bp, synthetic construct
  source 1..828: mol_type = other DNA
atgggcctgatgctgatcgactggtgtgccctggccctggtggtgttcatcggcctgccccacggcgccctggacgccgccatctctttctctatgatctcttctgccaagcgaatcgcccgactggccggcatcctgctgatctacctgctgctggccaccgccttcttcctgatctggtaccagctgcccgccttctctctgctgatcttcctgctgatctctatcatccacttcggcatggccgacttcaacgcctctccctctaagctgaagtggccccacatcatcgcccacggcggcgtggtgaccgtgtggctgcccctgatccagaagaacgaggtgaccaagctgttctctatcctgaccaacggccccacccccatcctgtgggacatcctgctgatcttcttcctgtgttggtctatcggcgtgtgtctgcacacctacgagaccctgcgatctaagcactacaacatcgccttcgagctgatcggcctgatcttcctggcctggtacgccccccccctggtgaccttcgccacctacttctgtttcatccactctcgacgacacttctctttcgtgtggaagcagctgcagcacatgtcttctaagaagatgatgatcggctctgccatcatcctgtcttgtacctcttggctgatcggcggcggcatctacttcttcctgaactctaagatgatcgcctctgaggccgccctgcagaccgtgttcatcggcctggccgccctgaccgtgccccacatgatcctgatcgacttcatcttccgaccccactcttctcgaatcaagatcaagaactag

SEQ ID NO: 13 - DNA, 1533 bp, synthetic construct
  source 1..1533: mol_type = other DNA
tgcctcctgtctgactcgtcattgccgcctttggagtacgactccaactatgagtgtgcttggatcactttgacgatacattcttcgttggaggctgtgggtctgacagctgcgttttcggcgcggttggccgacaacaatatcagctgcaacgtcattgctggctttcatcatgatcacatttttgtcggcaaaggcgacgcccagagagccattgacgttctttctaatttggaccgatagccgtatagtccagtctatctataagttcaactaactcgtaactattaccataacatatacttcactgccccagataaggttccgataaaaagttctgcagactaaatttatttcagtctcctcttcaccaccaaaatgccctcctacgaagctcgagctaacgtccacaagtccgcctttgccgctcgagtgctcaagctcgtggcagccaagaaaaccaacctgtgtgcttctctggatgttaccaccaccaaggagctcattgagcttgccgataaggtcggaccttatgtgtgcatgatcaagacccatatcgacatcattgacgacttcacctacgccggcactgtgctccccctcaaggaacttgctcttaagcacggtttcttcctgttcgaggacagaaagttcgcagatattggcaacactgtcaagcaccagtacaagaacggtgtctaccgaatcgccgagtggtccgatatcaccaacgcccacggtgtacccggaaccggaatcattgctggcctgcgagctggtgccgaggaaactgtctctgaacagaagaaggaggacgtctctgactacgagaactcccagtacaaggagttcctggtcccctctcccaacgagaagctggccagaggtctgctcatgctggccgagctgtcttgcaagggctctctggccactggcgagtactccaagcagaccattgagcttgcccgatccgaccccgagtttgtggttggcttcattgcccagaaccgacctaagggcgactctgaggactggcttattctgacccccggggtgggtcttgacgacaagggagacgctctcggacagcagtaccgaactgttgaggatgtcatgtctaccggaacggatatcataattgtcggccgaggtctgtacggccagaaccgagatcctattgaggaggccaagcgataccagaaggctggctgggaggcttaccagaagattaactgttagaggttagactatggatatgtcatttaactgtgtatatagagagcgtgcaagtatggagcgcttgttcagcttgtatgatggtcagacgacctgtctgatcgagtatgtatgatactgcacaacctgtgtatccgcatgatctgtccaatggggcatgttgttgtgtttctcgatacggagatgctgggtacaagtagctaatacgattgaactacttatacttatatgaggcttgaagaaagctgacttgtgtatgacttattctcaactacatccccagtcacaataccacca

SEQ ID NO: 14 - DNA, 30 bp, synthetic construct
  source 1..30: mol_type = other DNA
tcaccacccatcacgctcaatacccctgtg

SEQ ID NO: 15 - DNA, 44 bp, synthetic construct
  source 1..44: mol_type = other DNA
atgacgagtcagacaggaggcatgctgtgtgggttttgtaggtg

SEQ ID NO: 16 - DNA, 44 bp, synthetic construct
  source 1..44: mol_type = other DNA
cacctacaaaacccacacagcatgcctcctgtctgactcgtcat

SEQ ID NO: 17 - DNA, 44 bp, synthetic construct
  source 1..44: mol_type = other DNA
gatggatttggtgagtgcgagttggtggtattgtgactggggat

SEQ ID NO: 18 - DNA, 44 bp, synthetic construct
  source 1..44: mol_type = other DNA
atccccagtcacaataccaccaactcgcactcaccaaatccatc

SEQ ID NO: 19 - DNA, 44 bp, synthetic construct
  source 1..44: mol_type = other DNA
gtaaaacacccgtcaactagaatgctgtgtgggttttgtaggtg

SEQ ID NO: 20 - DNA, 44 bp, synthetic construct
  source 1..44: mol_type = other DNA
cacctacaaaacccacacagcattctagttgacgggtgttttac

SEQ ID NO: 21 - DNA, 30 bp, synthetic construct
  source 1..30: mol_type = other DNA
atgccaccccgctcagcttggaaccttcac

SEQ ID NO: 22 - DNA, 24 bp, synthetic construct
  source 1..24: mol_type = other DNA
tatctggggtatgacgggaaacgg

SEQ ID NO: 23 - DNA, 24 bp, synthetic construct
  source 1..24: mol_type = other DNA
agcccattttgtgcaacgacacat

SEQ ID NO: 24 - DNA, 30 bp, synthetic construct
  source 1..30: mol_type = other DNA
ctctgacgcggtttagagcctaccgaggcg

SEQ ID NO: 25 - DNA, 44 bp, synthetic construct
  source 1..44: mol_type = other DNA
atgacgagtcagacaggaggcaaatgattaatgaatgtgtacta

SEQ ID NO: 26 - DNA, 44 bp, synthetic construct
  source 1..44: mol_type = other DNA
tagtacacattcattaatcatttgcctcctgtctgactcgtcat

SEQ ID NO: 27 - DNA, 44 bp, synthetic construct
  source 1..44: mol_type = other DNA
gtgtcaaaaaaacgagatccattggtggtattgtgactggggat

SEQ ID NO: 28 - DNA, 44 bp, synthetic construct
  source 1..44: mol_type = other DNA
atccccagtcacaataccaccaatggatctcgtttttttgacac

SEQ ID NO: 29 - DNA, 44 bp, synthetic construct
  source 1..44: mol_type = other DNA
aacaaataattattcaatacaaaatgattaatgaatgtgtacta

SEQ ID NO: 30 - DNA, 40 bp, synthetic construct
  source 1..40: mol_type = other DNA
tagtacacattcattaatcattttgtattgaataattatt

SEQ ID NO: 31 - DNA, 30 bp, synthetic construct
  source 1..30: mol_type = other DNA
caccgtgcacacctcgtggctcccttgaaa

SEQ ID NO: 32 - DNA, 24 bp, synthetic construct
  source 1..24: mol_type = other DNA
tgtttacttacaagttgaatggtc

SEQ ID NO: 33 - DNA, 25 bp, synthetic construct
  source 1..25: mol_type = other DNA
aatccaccttggctgggtgctctac

SEQ ID NO: 34 - DNA, 30 bp, synthetic construct
  source 1..30: mol_type = other DNA
ccgattttaaatttcacttacacttcactt

SEQ ID NO: 35 - DNA, 44 bp, synthetic construct
  source 1..44: mol_type = other DNA
atgacgagtcagacaggaggcatttgtactgggtgatgcaaacg

SEQ ID NO: 36 - DNA, 44 bp, synthetic construct
  source 1..44: mol_type = other DNA
cgtttgcatcacccagtacaaatgcctcctgtctgactcgtcat

SEQ ID NO: 37 - DNA, 44 bp, synthetic construct
  source 1..44: mol_type = other DNA
ctgtactgggactcatcggggatggtggtattgtgactggggat

SEQ ID NO: 38 - DNA, 44 bp, synthetic construct
  source 1..44: mol_type = other DNA
atccccagtcacaataccaccatccccgatgagtcccagtacag

SEQ ID NO: 39 - DNA, 44 bp, synthetic construct
  source 1..44: mol_type = other DNA
cgctgcgaggatatcacttagctttgtactgggtgatgcaaacg

SEQ ID NO: 40 - DNA, 44 bp, synthetic construct
  source 1..44: mol_type = other DNA
cgtttgcatcacccagtacaaagctaagtgatatcctcgcagcg

SEQ ID NO: 41 - DNA, 30 bp, synthetic construct
  source 1..30: mol_type = other DNA
ctggtacatgtaggagttctttcgcccctg

SEQ ID NO: 42 - DNA, 23 bp, synthetic construct
  source 1..23: mol_type = other DNA
cgttgttatggagacgcgaagta

SEQ ID NO: 43 - DNA, 24 bp, synthetic construct
  source 1..24: mol_type = other DNA
gttctggttatataccggagagta